European Patent Specification EP 3 245 291 B1, published February 25, 2026. Title: Novel Micro-Dystrophins and Related Methods of Use. Applicant: Chamberlain, Jeffrey S. Ramos, Julian Hauschka, Stephen D. The sequence listing filed with the application follows.

SEQUENCE LISTING (22 sequences)

SEQ ID NO: 1 - DNA, 455 bp, Artificial Sequence
  hum-cTnT455
ctgctcccagctggccctcccaggcctgggttgctggcctctgctttatcaggattctcaagagggacagctggtttatgttgcatgactgttccctgcatatctgctctggttttaaatagcttatctgctagcctgctcccagctggccctcccaggcctgggttgctggcctctgctttatcaggattctcaagagggacagctggtttatgttgcatgactgttccctgcatatctgctctggttttaaatagcttatctgagcagctggaggaccacatgggcttatatggggcacctgccaaaatagcagccaacacccccccctgtcgcacattcctccctggctcaccaggccccagcccacatgcctgcttaaagccctctccatcctctgcctcacccagtccccgctgagactgagcagacgcctccaggatctgtcggcagct

SEQ ID NO: 2 - DNA, 495 bp, Homo sapiens
agttcaagtggagcagcacataactcttgccctctgccttccaagattctggtgctgagacttatggagtgtcttggaggttgccttctgccccccaaccctgctcccagctggccctcccaggcctgggttgctggcctctgctttatcaggattctcaagagggacagctggtttatgttgcatgactgttccctgcatatctgctctggttttaaatagcttatctgagcagctggaggaccacatgggcttatatggcgtggggtacatgttcctgtagccttgtccctggcacctgccaaaatagcagccaacaccccccacccccaccgccatccccctgccccacccgtcccctgtcgcacattcctccctccgcagggctggctcaccaggccccagcccacatgcctgcttaaagccctctccatcctctgcctcacccagtccccgctgagactgagcagacgcctccaggatctgtcggcagct

SEQ ID NO: 3 - protein, 1188 aa, Artificial Sequence
  micro-DysH3
MLWWEEVEDCYEREDVQKKTFTKWVNAQFSKFGKQHIENLFSDLQDGRRLLDLLEGLTGQKLPKEKGSTRVHALNNVNKALRVLQNNNVDLVNIGSTDIVDGNHKLTLGLIWNIILHWQVKNVMKNIMAGLQQTNSEKILLSWVRQSTRNYPQVNVINFTTSWSDGLALNALIHSHRPDLFDWNSVVCQQSATQRLEHAFNIARYQLGIEKLLDPEDVDTTYPDKKSILMYITSLFQVLPQQVSIEAIQEVEMLPRPPKVTKEEHFQLHHQMHYSQQITVSLAQGYERTSSPKPRFKSYAYTQAAYVTTSDPTRSPFPSQHLEAPEDKSFGSSLMESEVNLDRYQTALEEVLSWLLSAEDTLQAQGEISNDVEVVKDQFHTHEGYMMDLTAHQGRVGNILQLGSKLIGTGKLSEDEETEVQEQMNLLNSRWECLRVASMEKQSNLHRVLMDLQNQKLKELNDWLTKTEERTRKMEEEPLGPDLEDLKRQVQQHKVLQEDLEQEQVRVNSLTHMVVVVDESSGDHATAALEEQLKVLGDRWANICRWTEDRWVLLQDILLKWQRLTEEQCLFSAWLSEKEDAVNKIHTTGFKDQNEMLSSLQKLAVLKADLEKKKQSMGKLYSLKQDLLSTLKNKSVTQKTEAWLDNFARCWDNLVQKLEKSTAQISQAAPGLTTIGASPTQTVTLVTQPVVTKETAISKLEMPSSLMLELERLQELQEATDELDLKLRQAEVIKGSWQPVGDLLIDSLQDHLEKVKALRGEIAPLKENVSHVNDLARQLTTLGIQLSPYNLSTLEDLNTRWKLLQVAVEDRVRQLHEAHRDFGPASQHFLSTSVQGPWERAISPNKVPYYINHETQTTCWDHPKMTELYQSLADLNNVRFSAYRTAMKLRRLQKALCLDLLSLSAACDALDQHNLKQNDQPMDILQIINCLTTIYDRLEQEHNNLVNVPLCVDMCLNWLLNVYDTGRTGRIRVLSFKTGIISLCKAHLEDKYRYLFKQVASSTGFCDQRRLGLLLHDSIQIPRQLGEVASFGGSNIEPSVRSCFQFANNKPEIEAALFLDWMRLEPQSMVWLPVLHRVAAAETAKHQAKCNICKECPIIGFRYRSLKHFNYDICQSCFFSGRVAKGHKMHYPMVEYCTPTTSGEDVRDFAKVLKNKFRTKRYFAKHPRMGYLPVQTVLEGDNMETDTM

SEQ ID NO: 4 - protein, 1270 aa, Artificial Sequence
  micro-Dys5
MLWWEEVEDCYEREDVQKKTFTKWVNAQFSKFGKQHIENLFSDLQDGRRLLDLLEGLTGQKLPKEKGSTRVHALNNVNKALRVLQNNNVDLVNIGSTDIVDGNHKLTLGLIWNIILHWQVKNVMKNIMAGLQQTNSEKILLSWVRQSTRNYPQVNVINFTTSWSDGLALNALIHSHRPDLFDWNSVVCQQSATQRLEHAFNIARYQLGIEKLLDPEDVDTTYPDKKSILMYITSLFQVLPQQVSIEAIQEVEMLPRPPKVTKEEHFQLHHQMHYSQQITVSLAQGYERTSSPKPRFKSYAYTQAAYVTTSDPTRSPFPSQHLEAPEDKSFGSSLMESEVNLDRYQTALEEVLSWLLSAEDTLQAQGEISNDVEVVKDQFHTHEGYMMDLTAHQGRVGNILQLGSKLIGTGKLSEDEETEVQEQMNLLNSRWECLRVASMEKQSNLHSYVPSTYLTEITHVSQALLEVEQLLNAPDLCAKDFEDLFKQEESLKNIKDSLQQSSGRIDIIHSKKTAALQSATPVERVKLQEALSQLDFQWEKVNKMYKDRQGRFDRSVEKWRRFHYDIKIFNQWLTEAEQFLRKTQIPENWEHAKYKWYLKELQDGIGQRQTVVRTLNATGEEIIQQSSKTDASILQEKLGSLNLRWQEVCKQLSDRKKRLEEQSDQWKRLHLSLQELLVWLQLKDDELSRQAPIGGDFPAVQKQNDVHRAFKRELKTKEPVIMSTLETVRIFLTEQPLEGLEKLYQEPRELPPEERAQNVTRLLRKQAEEVNTEWEKLNLHSADWQRKIDETLERLQELQEATDELDLKLRQAEVIKGSWQPVGDLLIDSLQDHLEKVKALRGEIAPLKENVSHVNDLARQLTTLGIQLSPYNLSTLEDLNTRWKLLQVAVEDRVRQLHEAHRDFGPASQHFLSTSVQGPWERAISPNKVPYYINHETQTTCWDHPKMTELYQSLADLNNVRFSAYRTAMKLRRLQKALCLDLLSLSAACDALDQHNLKQNDQPMDILQIINCLTTIYDRLEQEHNNLVNVPLCVDMCLNWLLNVYDTGRTGRIRVLSFKTGIISLCKAHLEDKYRYLFKQVASSTGFCDQRRLGLLLHDSIQIPRQLGEVASFGGSNIEPSVRSCFQFANNKPEIEAALFLDWMRLEPQSMVWLPVLHRVAAAETAKHQAKCNICKECPIIGFRYRSLKHFNYDICQSCFFSGRVAKGHKMHYPMVEYCTPTTSGEDVRDFAKVLKNKFRTKRYFAKHPRMGYLPVQTVLEGDNMETDTM

SEQ ID NO: 5 - protein, 1404 aa, Artificial Sequence
  micro-Dys7
MLWWEEVEDCYEREDVQKKTFTKWVNAQFSKFGKQHIENLFSDLQDGRRLLDLLEGLTGQKLPKEKGSTRVHALNNVNKALRVLQNNNVDLVNIGSTDIVDGNHKLTLGLIWNIILHWQVKNVMKNIMAGLQQTNSEKILLSWVRQSTRNYPQVNVINFTTSWSDGLALNALIHSHRPDLFDWNSVVCQQSATQRLEHAFNIARYQLGIEKLLDPEDVDTTYPDKKSILMYITSLFQVLPQQVSIEAIQEVEMLPRPPKVTKEEHFQLHHQMHYSQQITVSLAQGYERTSSPKPRFKSYAYTQAAYVTTSDPTRSPFPSQHLEAPEDKSFGSSLMESEVNLDRYQTALEEVLSWLLSAEDTLQAQGEISNDVEVVKDQFHTHEGYMMDLTAHQGRVGNILQLGSKLIGTGKLSEDEETEVQEQMNLLNSRWECLRVASMEKQSNLHRVLMDLQNQKLKELNDWLTKTEERTRKMEEEPLGPDLEDLKRQVQQHKVLQEDLEQEQVRVNSLTHMVVVVDESSGDHATAALEEQLKVLGDRWANICRWTEDRWVLLQDILLKWQRLTEEQCLFSAWLSEKEDAVNKIHTTGFKDQNEMLSSLQKLAVLKADLEKKKQSMGKLYSLKQDLLSTLKNKSVTQKTEAWLDNFARCWDNLVQKLEKSTAQISQAAPGLTTIGASPTQTVTLVTQPVVTKETAISKLEMPSSLMLESYVPSTYLTEITHVSQALLEVEQLLNAPDLCAKDFEDLFKQEESLKNIKDSLQQSSGRIDIIHSKKTAALQSATPVERVKLQEALSQLDFQWEKVNKMYKDRQGRFDRSVEKWRRFHYDIKIFNQWLTEAEQFLRKTQIPENWEHAKYKWYLKELQDGIGQRQTVVRTLNATGEEIIQQSSKTDASILQEKLGSLNLRWQEVCKQLSDRKKRLEEQLERLQELQEATDELDLKLRQAEVIKGSWQPVGDLLIDSLQDHLEKVKALRGEIAPLKENVSHVNDLARQLTTLGIQLSPYNLSTLEDLNTRWKLLQVAVEDRVRQLHEAHRDFGPASQHFLSTSVQGPWERAISPNKVPYYINHETQTTCWDHPKMTELYQSLADLNNVRFSAYRTAMKLRRLQKALCLDLLSLSAACDALDQHNLKQNDQPMDILQIINCLTTIYDRLEQEHNNLVNVPLCVDMCLNWLLNVYDTGRTGRIRVLSFKTGIISLCKAHLEDKYRYLFKQVASSTGFCDQRRLGLLLHDSIQIPRQLGEVASFGGSNIEPSVRSCFQFANNKPEIEAALFLDWMRLEPQSMVWLPVLHRVAAAETAKHQAKCNICKECPIIGFRYRSLKHFNYDICQSCFFSGRVAKGHKMHYPMVEYCTPTTSGEDVRDFAKVLKNKFRTKRYFAKHPRMGYLPVQTVLEGDNMETDTM

SEQ ID NO: 6 - protein, 1190 aa, Artificial Sequence
  micro-Dys1
MLWWEEVEDCYEREDVQKKTFTKWVNAQFSKFGKQHIENLFSDLQDGRRLLDLLEGLTGQKLPKEKGSTRVHALNNVNKALRVLQNNNVDLVNIGSTDIVDGNHKLTLGLIWNIILHWQVKNVMKNIMAGLQQTNSEKILLSWVRQSTRNYPQVNVINFTTSWSDGLALNALIHSHRPDLFDWNSVVCQQSATQRLEHAFNIARYQLGIEKLLDPEDVDTTYPDKKSILMYITSLFQVLPQQVSIEAIQEVEMLPRPPKVTKEEHFQLHHQMHYSQQITVSLAQGYERTSSPKPRFKSYAYTQAAYVTTSDPTRSPFPSQHLEAPEDKSFGSSLMESEVNLDRYQTALEEVLSWLLSAEDTLQAQGEISNDVEVVKDQFHTHEGYMMDLTAHQGRVGNILQLGSKLIGTGKLSEDEETEVQEQMNLLNSRWECLRVASMEKQSNLHRVLMDLQNQKLKELNDWLTKTEERTRKMEEEPLGPDLEDLKRQVQQHKVLQEDLEQEQVRVNSLTHMVVVVDESSGDHATAALEEQLKVLGDRWANICRWTEDRWVLLQDILLKWQRLTEEQCLFSAWLSEKEDAVNKIHTTGFKDQNEMLSSLQKLAVLKADLEKKKQSMGKLYSLKQDLLSTLKNKSVTQKTEAWLDNFARCWDNLVQKLEKSTAQISQAELPPEERAQNVTRLLRKQAEEVNTEWEKLNLHSADWQRKIDETLERLQELQEATDELDLKLRQAEVIKGSWQPVGDLLIDSLQDHLEKVKALRGEIAPLKENVSHVNDLARQLTTLGIQLSPYNLSTLEDLNTRWKLLQVAVEDRVRQLHEAHRDFGPASQHFLSTSVQGPWERAISPNKVPYYINHETQTTCWDHPKMTELYQSLADLNNVRFSAYRTAMKLRRLQKALCLDLLSLSAACDALDQHNLKQNDQPMDILQIINCLTTIYDRLEQEHNNLVNVPLCVDMCLNWLLNVYDTGRTGRIRVLSFKTGIISLCKAHLEDKYRYLFKQVASSTGFCDQRRLGLLLHDSIQIPRQLGEVASFGGSNIEPSVRSCFQFANNKPEIEAALFLDWMRLEPQSMVWLPVLHRVAAAETAKHQAKCNICKECPIIGFRYRSLKHFNYDICQSCFFSGRVAKGHKMHYPMVEYCTPTTSGEDVRDFAKVLKNKFRTKRYFAKHPRMGYLPVQTVLEGDNMETDTM

SEQ ID NO: 7 - protein, 1184 aa, Artificial Sequence
  micro-Dys2
MLWWEEVEDCYEREDVQKKTFTKWVNAQFSKFGKQHIENLFSDLQDGRRLLDLLEGLTGQKLPKEKGSTRVHALNNVNKALRVLQNNNVDLVNIGSTDIVDGNHKLTLGLIWNIILHWQVKNVMKNIMAGLQQTNSEKILLSWVRQSTRNYPQVNVINFTTSWSDGLALNALIHSHRPDLFDWNSVVCQQSATQRLEHAFNIARYQLGIEKLLDPEDVDTTYPDKKSILMYITSLFQVLPQQVSIEAIQEVEMLPRPPKVTKEEHFQLHHQMHYSQQITVSLAQGYERTSSPKPRFKSYAYTQAAYVTTSDPTRSPFPSQHLEAPEDKSFGSSLMESEVNLDRYQTALEEVLSWLLSAEDTLQAQGEISNDVEVVKDQFHTHEGYMMDLTAHQGRVGNILQLGSKLIGTGKLSEDEETEVQEQMNLLNSRWECLRVASMEKQSNLHSYVPSTYLTEITHVSQALLEVEQLLNAPDLCAKDFEDLFKQEESLKNIKDSLQQSSGRIDIIHSKKTAALQSATPVERVKLQEALSQLDFQWEKVNKMYKDRQGRFDRSVEKWRRFHYDIKIFNQWLTEAEQFLRKTQIPENWEHAKYKWYLKELQDGIGQRQTVVRTLNATGEEIIQQSSKTDASILQEKLGSLNLRWQEVCKQLSDRKKRLEEQELPPEERAQNVTRLLRKQAEEVNTEWEKLNLHSADWQRKIDETLERLQELQEATDELDLKLRQAEVIKGSWQPVGDLLIDSLQDHLEKVKALRGEIAPLKENVSHVNDLARQLTTLGIQLSPYNLSTLEDLNTRWKLLQVAVEDRVRQLHEAHRDFGPASQHFLSTSVQGPWERAISPNKVPYYINHETQTTCWDHPKMTELYQSLADLNNVRFSAYRTAMKLRRLQKALCLDLLSLSAACDALDQHNLKQNDQPMDILQIINCLTTIYDRLEQEHNNLVNVPLCVDMCLNWLLNVYDTGRTGRIRVLSFKTGIISLCKAHLEDKYRYLFKQVASSTGFCDQRRLGLLLHDSIQIPRQLGEVASFGGSNIEPSVRSCFQFANNKPEIEAALFLDWMRLEPQSMVWLPVLHRVAAAETAKHQAKCNICKECPIIGFRYRSLKHFNYDICQSCFFSGRVAKGHKMHYPMVEYCTPTTSGEDVRDFAKVLKNKFRTKRYFAKHPRMGYLPVQTVLEGDNMETDTM

SEQ ID NO: 8 - protein, 1188 aa, Artificial Sequence
  micro-Dys3
MLWWEEVEDCYEREDVQKKTFTKWVNAQFSKFGKQHIENLFSDLQDGRRLLDLLEGLTGQKLPKEKGSTRVHALNNVNKALRVLQNNNVDLVNIGSTDIVDGNHKLTLGLIWNIILHWQVKNVMKNIMAGLQQTNSEKILLSWVRQSTRNYPQVNVINFTTSWSDGLALNALIHSHRPDLFDWNSVVCQQSATQRLEHAFNIARYQLGIEKLLDPEDVDTTYPDKKSILMYITSLFQVLPQQVSIEAIQEVEMLPRPPKVTKEEHFQLHHQMHYSQQITVSLAQGYERTSSPKPRFKSYAYTQAAYVTTSDPTRSPFPSQHLEAPEDKSFGSSLMESEVNLDRYQTALEEVLSWLLSAEDTLQAQGEISNDVEVVKDQFHTHEGYMMDLTAHQGRVGNILQLGSKLIGTGKLSEDEETEVQEQMNLLNSRWECLRVASMEKQSNLHRVLMDLQNQKLKELNDWLTKTEERTRKMEEEPLGPDLEDLKRQVQQHKVLQEDLEQEQVRVNSLTHMVVVVDESSGDHATAALEEQLKVLGDRWANICRWTEDRWVLLQDILLKWQRLTEEQCLFSAWLSEKEDAVNKIHTTGFKDQNEMLSSLQKLAVLKADLEKKKQSMGKLYSLKQDLLSTLKNKSVTQKTEAWLDNFARCWDNLVQKLEKSTAQISQAAPGLTTIGASPTQTVTLVTQPVVTKETAISKLEMPSSLMLEVPALADFNRAWTELTDWLSLLDQVIKSWQPVGDLLIDSLQDHLEKVKALRGEIAPLKENVSHVNDLARQLTTLGIQLSPYNLSTLEDLNTRWKLLQVAVEDRVRQLHEAHRDFGPASQHFLSTSVQGPWERAISPNKVPYYINHETQTTCWDHPKMTELYQSLADLNNVRFSAYRTAMKLRRLQKALCLDLLSLSAACDALDQHNLKQNDQPMDILQIINCLTTIYDRLEQEHNNLVNVPLCVDMCLNWLLNVYDTGRTGRIRVLSFKTGIISLCKAHLEDKYRYLFKQVASSTGFCDQRRLGLLLHDSIQIPRQLGEVASFGGSNIEPSVRSCFQFANNKPEIEAALFLDWMRLEPQSMVWLPVLHRVAAAETAKHQAKCNICKECPIIGFRYRSLKHFNYDICQSCFFSGRVAKGHKMHYPMVEYCTPTTSGEDVRDFAKVLKNKFRTKRYFAKHPRMGYLPVQTVLEGDNMETDTM

SEQ ID NO: 9 - protein, 1231 aa, Artificial Sequence
  micro-Dys4
MLWWEEVEDCYEREDVQKKTFTKWVNAQFSKFGKQHIENLFSDLQDGRRLLDLLEGLTGQKLPKEKGSTRVHALNNVNKALRVLQNNNVDLVNIGSTDIVDGNHKLTLGLIWNIILHWQVKNVMKNIMAGLQQTNSEKILLSWVRQSTRNYPQVNVINFTTSWSDGLALNALIHSHRPDLFDWNSVVCQQSATQRLEHAFNIARYQLGIEKLLDPEDVDTTYPDKKSILMYITSLFQVLPQQVSIEAIQEVEMLPRPPKVTKEEHFQLHHQMHYSQQITVSLAQGYERTSSPKPRFKSYAYTQAAYVTTSDPTRSPFPSQHLEAPEDKSFGSSLMESEVNLDRYQTALEEVLSWLLSAEDTLQAQGEISNDVEVVKDQFHTHEGYMMDLTAHQGRVGNILQLGSKLIGTGKLSEDEETEVQEQMNLLNSRWECLRVASMEKQSNLHRVLMDLQNQKLKELNDWLTKTEERTRKMEEEPLGPDLEDLKRQVQQHKVLQEDLEQEQVRVNSLTHMVVVVDESSGDHATAALEEQLKVLGDRWANICRWTEDRWVLLQDILLKWQRLTEEQCLFSAWLSEKEDAVNKIHTTGFKDQNEMLSSLQKLAVLKADLEKKKQSMGKLYSLKQDLLSTLKNKSVTQKTEAWLDNFARCWDNLVQKLEKSTAQISQAAPGLTTIGASPTQTVTLVTQPVVTKETAISKLEMPSSLMLEELPPEERAQNVTRLLRKQAEEVNTEWEKLNLHSADWQRKIDETLERLQELQEATDELDLKLRQAEVIKGSWQPVGDLLIDSLQDHLEKVKALRGEIAPLKENVSHVNDLARQLTTLGIQLSPYNLSTLEDLNTRWKLLQVAVEDRVRQLHEAHRDFGPASQHFLSTSVQGPWERAISPNKVPYYINHETQTTCWDHPKMTELYQSLADLNNVRFSAYRTAMKLRRLQKALCLDLLSLSAACDALDQHNLKQNDQPMDILQIINCLTTIYDRLEQEHNNLVNVPLCVDMCLNWLLNVYDTGRTGRIRVLSFKTGIISLCKAHLEDKYRYLFKQVASSTGFCDQRRLGLLLHDSIQIPRQLGEVASFGGSNIEPSVRSCFQFANNKPEIEAALFLDWMRLEPQSMVWLPVLHRVAAAETAKHQAKCNICKECPIIGFRYRSLKHFNYDICQSCFFSGRVAKGHKMHYPMVEYCTPTTSGEDVRDFAKVLKNKFRTKRYFAKHPRMGYLPVQTVLEGDNMETDTM

SEQ ID NO: 10 - protein, 1383 aa, Artificial Sequence
  micro-Dys6
MLWWEEVEDCYEREDVQKKTFTKWVNAQFSKFGKQHIENLFSDLQDGRRLLDLLEGLTGQKLPKEKGSTRVHALNNVNKALRVLQNNNVDLVNIGSTDIVDGNHKLTLGLIWNIILHWQVKNVMKNIMAGLQQTNSEKILLSWVRQSTRNYPQVNVINFTTSWSDGLALNALIHSHRPDLFDWNSVVCQQSATQRLEHAFNIARYQLGIEKLLDPEDVDTTYPDKKSILMYITSLFQVLPQQVSIEAIQEVEMLPRPPKVTKEEHFQLHHQMHYSQQITVSLAQGYERTSSPKPRFKSYAYTQAAYVTTSDPTRSPFPSQHLEAPEDKSFGSSLMESEVNLDRYQTALEEVLSWLLSAEDTLQAQGEISNDVEVVKDQFHTHEGYMMDLTAHQGRVGNILQLGSKLIGTGKLSEDEETEVQEQMNLLNSRWECLRVASMEKQSNLHRVLMDLQNQKLKELNDWLTKTEERTRKMEEEPLGPDLEDLKRQVQQHKVLQEDLEQEQVRVNSLTHMVVVVDESSGDHATAALEEQLKVLGDRWANICRWTEDRWVLLQDILLKWQRLTEEQCLFSAWLSEKEDAVNKIHTTGFKDQNEMLSSLQKLAVLKADLEKKKQSMGKLYSLKQDLLSTLKNKSVTQKTEAWLDNFARCWDNLVQKLEKSTAQISQAIHTVREETMMVMTEDMPLEISYVPSTYLTEITHVSQALLEVEQLLNAPDLCAKDFEDLFKQEESLKNIKDSLQQSSGRIDIIHSKKTAALQSATPVERVKLQEALSQLDFQWEKVNKMYKDRQGRFDRSVEKWRRFHYDIKIFNQWLTEAEQFLRKTQIPENWEHAKYKWYLKELQDGIGQRQTVVRTLNATGEEIIQQSSKTDASILQEKLGSLNLRWQEVCKQLSDRKKRLEEQLERLQELQEATDELDLKLRQAEVIKGSWQPVGDLLIDSLQDHLEKVKALRGEIAPLKENVSHVNDLARQLTTLGIQLSPYNLSTLEDLNTRWKLLQVAVEDRVRQLHEAHRDFGPASQHFLSTSVQGPWERAISPNKVPYYINHETQTTCWDHPKMTELYQSLADLNNVRFSAYRTAMKLRRLQKALCLDLLSLSAACDALDQHNLKQNDQPMDILQIINCLTTIYDRLEQEHNNLVNVPLCVDMCLNWLLNVYDTGRTGRIRVLSFKTGIISLCKAHLEDKYRYLFKQVASSTGFCDQRRLGLLLHDSIQIPRQLGEVASFGGSNIEPSVRSCFQFANNKPEIEAALFLDWMRLEPQSMVWLPVLHRVAAAETAKHQAKCNICKECPIIGFRYRSLKHFNYDICQSCFFSGRVAKGHKMHYPMVEYCTPTTSGEDVRDFAKVLKNKFRTKRYFAKHPRMGYLPVQTVLEGDNMETDTM

SEQ ID NO: 11 - DNA, 3564 bp, Artificial Sequence
  micro-DysH3
atgctttggtgggaagaagtagaggactgttatgaaagagaagatgttcaaaagaaaacattcacaaaatgggtaaatgcacaattttctaagtttgggaagcagcatattgagaacctcttcagtgacctacaggatgggaggcgcctcctagacctcctcgaaggcctgacagggcaaaaactgccaaaagaaaaaggatccacaagagttcatgccctgaacaatgtcaacaaggcactgcgggttttgcagaacaataatgttgatttagtgaatattggaagtactgacatcgtagatggaaatcataaactgactcttggtttgatttggaatataatcctccactggcaggtcaaaaatgtaatgaaaaatatcatggctggattgcaacaaaccaacagtgaaaagattctcctgagctgggtccgacaatcaactcgtaattatccacaggttaatgtaatcaacttcaccaccagctggtctgatggcctggctttgaatgctctcatccatagtcataggccagacctatttgactggaatagtgtggtttgccagcagtcagccacacaacgactggaacatgcattcaacatcgccagatatcaattaggcatagagaaactactcgatcctgaagatgttgataccacctatccagataagaagtccatcttaatgtacatcacatcactcttccaagttttgcctcaacaagtgagcattgaagccatccaggaagtggaaatgttgccaaggccacctaaagtgactaaagaagaacattttcagttacatcatcaaatgcactattctcaacagatcacggtcagtctagcacagggatatgagagaacttcttcccctaagcctcgattcaagagctatgcctacacacaggctgcttatgtcaccacctctgaccctacacggagcccatttccttcacagcatttggaagctcctgaagacaagtcatttggcagttcattgatggagagtgaagtaaacctggaccgttatcaaacagctttagaagaagtattatcgtggcttctttctgctgaggacacattgcaagcacaaggagagatttctaatgatgtggaagtggtgaaagaccagtttcatactcatgaggggtacatgatggatttgacagcccatcagggccgggttggtaatattctacaattgggaagtaagctgattggaacaggaaaattatcagaagatgaagaaactgaagtacaagagcagatgaatctcctaaattcaagatgggaatgcctcagggtagctagcatggaaaaacaaagcaatttacatagagttttaatggatctccagaatcagaaactgaaagagttgaatgactggctaacaaaaacagaagaaagaacaaggaaaatggaggaagagcctcttggacctgatcttgaagacctaaaacgccaagtacaacaacataaggtgcttcaagaagatctagaacaagaacaagtcagggtcaattctctcactcacatggtggtggtagttgatgaatctagtggagatcacgcaactgctgctttggaagaacaacttaaggtattgggagatcgatgggcaaacatctgtagatggacagaagaccgctgggttcttttacaagacatccttctcaaatggcaacgtcttactgaagaacagtgcctttttagtgcatggctttcagaaaaagaagatgcagtgaacaagattcacacaactggctttaaagatcaaaatgaaatgttatcaagtcttcaaaaactggccgttttaaaagcggatctagaaaagaaaaagcaatccatgggcaaactgtattcactcaaacaagatcttctttcaacactgaagaataagtcagtgacccagaagacggaagcatggctggataactttgcccggtgttgggataatttagtccaaaaacttgaaaagagtacagcacagatttcacaggctgctcctggactgaccactattggagcctctcctactcagactgttactctggtgacacaacctgtggttactaaggaaactgccatctccaaactagaaatgccatcttccttgatgttggagcttgaaagactccaggaacttcaagaggccacggatgagctggacctcaagctgcgccaagctgaggtgatcaagggatcctggcagcccgtgggcgatctcctcattgactctctccaagatcacctcgagaaagtcaaggcacttcgaggagaaattgcgcctctgaaagagaacgtgagccacgtcaatgaccttgctcgccagcttaccactttgggcattcagctctcaccgtataacctcagcactctggaagacctgaacaccagatggaagcttctgcaggtggccgtcgaggaccgagtcaggcagctgcatgaagcccacagggactttggtccagcatctcagcactttctttccacgtctgtccagggtccctgggagagagccatctcgccaaacaaagtgccctactatatcaaccacgagactcaaacaacttgctgggaccatcccaaaatgacagagctctaccagtctttagctgacctgaataatgtcagattctcagcttataggactgccatgaaactccgaagactgcagaaggccctttgcttggatctcttgagcctgtcagctgcatgtgatgccttggaccagcacaacctcaagcaaaatgaccagcccatggatatcctgcagattattaattgtttgaccactatttatgaccgcctggagcaagagcacaacaatttggtcaacgtccctctctgcgtggatatgtgtctgaactggctgctgaatgtttatgatacgggacgaacagggaggatccgtgtcctgtcttttaaaactggcatcatttccctgtgtaaagcacatttggaagacaagtacagataccttttcaagcaagtggcaagttcaacaggattttgtgaccagcgcaggctgggcctccttctgcatgattctatccaaattccaagacagttgggtgaagttgcatcctttgggggcagtaacattgagccaagtgtccggagctgcttccaatttgctaataataagccagagatcgaagcggccctcttcctagactggatgagactggaaccccagtccatggtgtggctgcccgtcctgcacagagtggctgctgcagaaactgccaagcatcaggccaaatgtaacatctgcaaagagtgtccaatcattggattcaggtacaggagtctaaagcactttaattatgacatctgccaaagctgctttttttctggtcgagttgcaaaaggccataaaatgcactatcccatggtggaatattgcactccgactacatcaggagaagatgttcgagactttgccaaggtactaaaaaacaaatttcgaaccaaaaggtattttgcgaagcatccccgaatgggctacctgccagtgcagactgtcttagagggggacaacatggaaactgacacaatg

SEQ ID NO: 12 - DNA, 3570 bp, Artificial Sequence
  micro-Dys1
atgctttggtgggaagaagtagaggactgttatgaaagagaagatgttcaaaagaaaacattcacaaaatgggtaaatgcacaattttctaagtttgggaagcagcatattgagaacctcttcagtgacctacaggatgggaggcgcctcctagacctcctcgaaggcctgacagggcaaaaactgccaaaagaaaaaggatccacaagagttcatgccctgaacaatgtcaacaaggcactgcgggttttgcagaacaataatgttgatttagtgaatattggaagtactgacatcgtagatggaaatcataaactgactcttggtttgatttggaatataatcctccactggcaggtcaaaaatgtaatgaaaaatatcatggctggattgcaacaaaccaacagtgaaaagattctcctgagctgggtccgacaatcaactcgtaattatccacaggttaatgtaatcaacttcaccaccagctggtctgatggcctggctttgaatgctctcatccatagtcataggccagacctatttgactggaatagtgtggtttgccagcagtcagccacacaacgactggaacatgcattcaacatcgccagatatcaattaggcatagagaaactactcgatcctgaagatgttgataccacctatccagataagaagtccatcttaatgtacatcacatcactcttccaagttttgcctcaacaagtgagcattgaagccatccaggaagtggaaatgttgccaaggccacctaaagtgactaaagaagaacattttcagttacatcatcaaatgcactattctcaacagatcacggtcagtctagcacagggatatgagagaacttcttcccctaagcctcgattcaagagctatgcctacacacaggctgcttatgtcaccacctctgaccctacacggagcccatttccttcacagcatttggaagctcctgaagacaagtcatttggcagttcattgatggagagtgaagtaaacctggaccgttatcaaacagctttagaagaagtattatcgtggcttctttctgctgaggacacattgcaagcacaaggagagatttctaatgatgtggaagtggtgaaagaccagtttcatactcatgaggggtacatgatggatttgacagcccatcagggccgggttggtaatattctacaattgggaagtaagctgattggaacaggaaaattatcagaagatgaagaaactgaagtacaagagcagatgaatctcctaaattcaagatgggaatgcctcagggtagctagcatggaaaaacaaagcaatttacatagagttttaatggatctccagaatcagaaactgaaagagttgaatgactggctaacaaaaacagaagaaagaacaaggaaaatggaggaagagcctcttggacctgatcttgaagacctaaaacgccaagtacaacaacataaggtgcttcaagaagatctagaacaagaacaagtcagggtcaattctctcactcacatggtggtggtagttgatgaatctagtggagatcacgcaactgctgctttggaagaacaacttaaggtattgggagatcgatgggcaaacatctgtagatggacagaagaccgctgggttcttttacaagacatccttctcaaatggcaacgtcttactgaagaacagtgcctttttagtgcatggctttcagaaaaagaagatgcagtgaacaagattcacacaactggctttaaggatcaaaatgaaatgttatcaagtcttcaaaaactggccgttttaaaagcggatctagaaaagaaaaagcaatccatgggcaaactgtattcactcaaacaagatcttctttcaacactgaagaataagtcagtgacccagaagacggaagcatggctggataactttgcccggtgttgggataatttagtccaaaaacttgaaaagagtacagcacagatttcacaggctgagctgcctcctgaggagagagcccagaatgtcactcggcttctacgaaagcaggctgaggaggtcaatactgagtgggaaaaattgaacctgcactccgctgactggcagagaaaaatagatgagacccttgaaagactccaggaacttcaagaggccacggatgagctggacctcaagctgcgccaagctgaggtgatcaagggatcctggcagcccgtgggcgatctcctcattgactctctccaagatcacctcgagaaagtcaaggcacttcgaggagaaattgcgcctctgaaagagaacgtgagccacgtcaatgaccttgctcgccagcttaccactttgggcattcagctctcaccgtataacctcagcactctggaagacctgaacaccagatggaagcttctgcaggtggccgtcgaggaccgagtcaggcagctgcatgaagcccacagggactttggtccagcatctcagcactttctttccacgtctgtccagggtccctgggagagagccatctcgccaaacaaagtgccctactatatcaaccacgagactcaaacaacttgctgggaccatcccaaaatgacagagctctaccagtctttagctgacctgaataatgtcagattctcagcttataggactgccatgaaactccgaagactgcagaaggccctttgcttggatctcttgagcctgtcagctgcatgtgatgccttggaccagcacaacctcaagcaaaatgaccagcccatggatatcctgcagattattaattgtttgaccactatttatgaccgcctggagcaagagcacaacaatttggtcaacgtccctctctgcgtggatatgtgtctgaactggctgctgaatgtttatgatacgggacgaacagggaggatccgtgtcctgtcttttaaaactggcatcatttccctgtgtaaagcacatttggaagacaagtacagataccttttcaagcaagtggcaagttcaacaggattttgtgaccagcgcaggctgggcctccttctgcatgattctatccaaattccaagacagttgggtgaagttgcatcctttgggggcagtaacattgagccaagtgtccggagctgcttccaatttgctaataataagccagagatcgaagcggccctcttcctagactggatgagactggaaccccagtccatggtgtggctgcccgtcctgcacagagtggctgctgcagaaactgccaagcatcaggccaaatgtaacatctgcaaagagtgtccaatcattggattcaggtacaggagtctaaagcactttaattatgacatctgccaaagctgctttttttctggtcgagttgcaaaaggccataaaatgcactatcccatggtggaatattgcactccgactacatcaggagaagatgttcgagactttgccaaggtactaaaaaacaaatttcgaaccaaaaggtattttgcgaagcatccccgaatgggctacctgccagtgcagactgtcttagagggggacaacatggaaactgacacaatg

SEQ ID NO: 13 - DNA, 3552 bp, Artificial Sequence
  micro-Dys2
atgctttggtgggaagaagtagaggactgttatgaaagagaagatgttcaaaagaaaacattcacaaaatgggtaaatgcacaattttctaagtttgggaagcagcatattgagaacctcttcagtgacctacaggatgggaggcgcctcctagacctcctcgaaggcctgacagggcaaaaactgccaaaagaaaaaggatccacaagagttcatgccctgaacaatgtcaacaaggcactgcgggttttgcagaacaataatgttgatttagtgaatattggaagtactgacatcgtagatggaaatcataaactgactcttggtttgatttggaatataatcctccactggcaggtcaaaaatgtaatgaaaaatatcatggctggattgcaacaaaccaacagtgaaaagattctcctgagctgggtccgacaatcaactcgtaattatccacaggttaatgtaatcaacttcaccaccagctggtctgatggcctggctttgaatgctctcatccatagtcataggccagacctatttgactggaatagtgtggtttgccagcagtcagccacacaacgactggaacatgcattcaacatcgccagatatcaattaggcatagagaaactactcgatcctgaagatgttgataccacctatccagataagaagtccatcttaatgtacatcacatcactcttccaagttttgcctcaacaagtgagcattgaagccatccaggaagtggaaatgttgccaaggccacctaaagtgactaaagaagaacattttcagttacatcatcaaatgcactattctcaacagatcacggtcagtctagcacagggatatgagagaacttcttcccctaagcctcgattcaagagctatgcctacacacaggctgcttatgtcaccacctctgaccctacacggagcccatttccttcacagcatttggaagctcctgaagacaagtcatttggcagttcattgatggagagtgaagtaaacctggaccgttatcaaacagctttagaagaagtattatcgtggcttctttctgctgaggacacattgcaagcacaaggagagatttctaatgatgtggaagtggtgaaagaccagtttcatactcatgaggggtacatgatggatttgacagcccatcagggccgggttggtaatattctacaattgggaagtaagctgattggaacaggaaaattatcagaagatgaagaaactgaagtacaagagcagatgaatctcctaaattcaagatgggaatgcctcagggtagctagcatggaaaaacaaagcaatttacattcttatgtgccttctacttatttgactgaaatcactcatgtctcacaagccctattagaagtggaacaacttctcaatgctcctgacctctgtgctaaggactttgaagatctctttaagcaagaggagtctctgaagaatataaaagatagtctacaacaaagctcaggtcggattgacattattcatagcaagaagacagcagcattgcaaagtgcaacgcctgtggaaagggtgaagctacaggaagctctctcccagcttgatttccaatgggaaaaagttaacaaaatgtacaaggaccgacaagggcgatttgacagatctgttgagaaatggcggcgttttcattatgatataaagatatttaatcagtggctaacagaagctgaacagtttctcagaaagacacaaattcctgagaattgggaacatgctaaatacaaatggtatcttaaggaactccaggatggcattgggcagcggcaaactgttgtcagaacattgaatgcaactggggaagaaataattcagcaatcctcaaaaacagatgccagtattctacaggaaaaattgggaagcctgaatctgcggtggcaggaggtctgcaaacagctgtcagacagaaaaaagaggctagaagaacaagagctgcctcctgaggagagagcccagaatgtcactcggcttctacgaaagcaggctgaggaggtcaatactgagtgggaaaaattgaacctgcactccgctgactggcagagaaaaatagatgagacccttgaaagactccaggaacttcaagaggccacggatgagctggacctcaagctgcgccaagctgaggtgatcaagggatcctggcagcccgtgggcgatctcctcattgactctctccaagatcacctcgagaaagtcaaggcacttcgaggagaaattgcgcctctgaaagagaacgtgagccacgtcaatgaccttgctcgccagcttaccactttgggcattcagctctcaccgtataacctcagcactctggaagacctgaacaccagatggaagcttctgcaggtggccgtcgaggaccgagtcaggcagctgcatgaagcccacagggactttggtccagcatctcagcactttctttccacgtctgtccagggtccctgggagagagccatctcgccaaacaaagtgccctactatatcaaccacgagactcaaacaacttgctgggaccatcccaaaatgacagagctctaccagtctttagctgacctgaataatgtcagattctcagcttataggactgccatgaaactccgaagactgcagaaggccctttgcttggatctcttgagcctgtcagctgcatgtgatgccttggaccagcacaacctcaagcaaaatgaccagcccatggatatcctgcagattattaattgtttgaccactatttatgaccgcctggagcaagagcacaacaatttggtcaacgtccctctctgcgtggatatgtgtctgaactggctgctgaatgtttatgatacgggacgaacagggaggatccgtgtcctgtcttttaaaactggcatcatttccctgtgtaaagcacatttggaagacaagtacagataccttttcaagcaagtggcaagttcaacaggattttgtgaccagcgcaggctgggcctccttctgcatgattctatccaaattccaagacagttgggtgaagttgcatcctttgggggcagtaacattgagccaagtgtccggagctgcttccaatttgctaataataagccagagatcgaagcggccctcttcctagactggatgagactggaaccccagtccatggtgtggctgcccgtcctgcacagagtggctgctgcagaaactgccaagcatcaggccaaatgtaacatctgcaaagagtgtccaatcattggattcaggtacaggagtctaaagcactttaattatgacatctgccaaagctgctttttttctggtcgagttgcaaaaggccataaaatgcactatcccatggtggaatattgcactccgactacatcaggagaagatgttcgagactttgccaaggtactaaaaaacaaatttcgaaccaaaaggtattttgcgaagcatccccgaatgggctacctgccagtgcagactgtcttagagggggacaacatggaaactgacacaatg

SEQ ID NO: 14 - DNA, 3564 bp, Artificial Sequence
  micro-Dys3
atgctttggtgggaagaagtagaggactgttatgaaagagaagatgttcaaaagaaaacattcacaaaatgggtaaatgcacaattttctaagtttgggaagcagcatattgagaacctcttcagtgacctacaggatgggaggcgcctcctagacctcctcgaaggcctgacagggcaaaaactgccaaaagaaaaaggatccacaagagttcatgccctgaacaatgtcaacaaggcactgcgggttttgcagaacaataatgttgatttagtgaatattggaagtactgacatcgtagatggaaatcataaactgactcttggtttgatttggaatataatcctccactggcaggtcaaaaatgtaatgaaaaatatcatggctggattgcaacaaaccaacagtgaaaagattctcctgagctgggtccgacaatcaactcgtaattatccacaggttaatgtaatcaacttcaccaccagctggtctgatggcctggctttgaatgctctcatccatagtcataggccagacctatttgactggaatagtgtggtttgccagcagtcagccacacaacgactggaacatgcattcaacatcgccagatatcaattaggcatagagaaactactcgatcctgaagatgttgataccacctatccagataagaagtccatcttaatgtacatcacatcactcttccaagttttgcctcaacaagtgagcattgaagccatccaggaagtggaaatgttgccaaggccacctaaagtgactaaagaagaacattttcagttacatcatcaaatgcactattctcaacagatcacggtcagtctagcacagggatatgagagaacttcttcccctaagcctcgattcaagagctatgcctacacacaggctgcttatgtcaccacctctgaccctacacggagcccatttccttcacagcatttggaagctcctgaagacaagtcatttggcagttcattgatggagagtgaagtaaacctggaccgttatcaaacagctttagaagaagtattatcgtggcttctttctgctgaggacacattgcaagcacaaggagagatttctaatgatgtggaagtggtgaaagaccagtttcatactcatgaggggtacatgatggatttgacagcccatcagggccgggttggtaatattctacaattgggaagtaagctgattggaacaggaaaattatcagaagatgaagaaactgaagtacaagagcagatgaatctcctaaattcaagatgggaatgcctcagggtagctagcatggaaaaacaaagcaatttacatagagttttaatggatctccagaatcagaaactgaaagagttgaatgactggctaacaaaaacagaagaaagaacaaggaaaatggaggaagagcctcttggacctgatcttgaagacctaaaacgccaagtacaacaacataaggtgcttcaagaagatctagaacaagaacaagtcagggtcaattctctcactcacatggtggtggtagttgatgaatctagtggagatcacgcaactgctgctttggaagaacaacttaaggtattgggagatcgatgggcaaacatctgtagatggacagaagaccgctgggttcttttacaagacatccttctcaaatggcaacgtcttactgaagaacagtgcctttttagtgcatggctttcagaaaaagaagatgcagtgaacaagattcacacaactggctttaaagatcaaaatgaaatgttatcaagtcttcaaaaactggccgttttaaaagcggatctagaaaagaaaaagcaatccatgggcaaactgtattcactcaaacaagatcttctttcaacactgaagaataagtcagtgacccagaagacggaagcatggctggataactttgcccggtgttgggataatttagtccaaaaacttgaaaagagtacagcacagatttcacaggctgctcctggactgaccactattggagcctctcctactcagactgttactctggtgacacaacctgtggttactaaggaaactgccatctccaaactagaaatgccatcttccttgatgttggaggtacctgctctggcagatttcaaccgggcttggacagaacttaccgactggctttctctgcttgatcaagttataaaatcatggcagcccgtgggcgatctcctcattgactctctccaagatcacctcgagaaagtcaaggcacttcgaggagaaattgcgcctctgaaagagaacgtgagccacgtcaatgaccttgctcgccagcttaccactttgggcattcagctctcaccgtataacctcagcactctggaagacctgaacaccagatggaagcttctgcaggtggccgtcgaggaccgagtcaggcagctgcatgaagcccacagggactttggtccagcatctcagcactttctttccacgtctgtccagggtccctgggagagagccatctcgccaaacaaagtgccctactatatcaaccacgagactcaaacaacttgctgggaccatcccaaaatgacagagctctaccagtctttagctgacctgaataatgtcagattctcagcttataggactgccatgaaactccgaagactgcagaaggccctttgcttggatctcttgagcctgtcagctgcatgtgatgccttggaccagcacaacctcaagcaaaatgaccagcccatggatatcctgcagattattaattgtttgaccactatttatgaccgcctggagcaagagcacaacaatttggtcaacgtccctctctgcgtggatatgtgtctgaactggctgctgaatgtttatgatacgggacgaacagggaggatccgtgtcctgtcttttaaaactggcatcatttccctgtgtaaagcacatttggaagacaagtacagataccttttcaagcaagtggcaagttcaacaggattttgtgaccagcgcaggctgggcctccttctgcatgattctatccaaattccaagacagttgggtgaagttgcatcctttgggggcagtaacattgagccaagtgtccggagctgcttccaatttgctaataataagccagagatcgaagcggccctcttcctagactggatgagactggaaccccagtccatggtgtggctgcccgtcctgcacagagtggctgctgcagaaactgccaagcatcaggccaaatgtaacatctgcaaagagtgtccaatcattggattcaggtacaggagtctaaagcactttaattatgacatctgccaaagctgctttttttctggtcgagttgcaaaaggccataaaatgcactatcccatggtggaatattgcactccgactacatcaggagaagatgttcgagactttgccaaggtactaaaaaacaaatttcgaaccaaaaggtattttgcgaagcatccccgaatgggctacctgccagtgcagactgtcttagagggggacaacatggaaactgacacaatg

SEQ ID NO: 15 - DNA, 3693 bp, Artificial Sequence
  micro-Dys4
atgctttggtgggaagaagtagaggactgttatgaaagagaagatgttcaaaagaaaacattcacaaaatgggtaaatgcacaattttctaagtttgggaagcagcatattgagaacctcttcagtgacctacaggatgggaggcgcctcctagacctcctcgaaggcctgacagggcaaaaactgccaaaagaaaaaggatccacaagagttcatgccctgaacaatgtcaacaaggcactgcgggttttgcagaacaataatgttgatttagtgaatattggaagtactgacatcgtagatggaaatcataaactgactcttggtttgatttggaatataatcctccactggcaggtcaaaaatgtaatgaaaaatatcatggctggattgcaacaaaccaacagtgaaaagattctcctgagctgggtccgacaatcaactcgtaattatccacaggttaatgtaatcaacttcaccaccagctggtctgatggcctggctttgaatgctctcatccatagtcataggccagacctatttgactggaatagtgtggtttgccagcagtcagccacacaacgactggaacatgcattcaacatcgccagatatcaattaggcatagagaaactactcgatcctgaagatgttgataccacctatccagataagaagtccatcttaatgtacatcacatcactcttccaagttttgcctcaacaagtgagcattgaagccatccaggaagtggaaatgttgccaaggccacctaaagtgactaaagaagaacattttcagttacatcatcaaatgcactattctcaacagatcacggtcagtctagcacagggatatgagagaacttcttcccctaagcctcgattcaagagctatgcctacacacaggctgcttatgtcaccacctctgaccctacacggagcccatttccttcacagcatttggaagctcctgaagacaagtcatttggcagttcattgatggagagtgaagtaaacctggaccgttatcaaacagctttagaagaagtattatcgtggcttctttctgctgaggacacattgcaagcacaaggagagatttctaatgatgtggaagtggtgaaagaccagtttcatactcatgaggggtacatgatggatttgacagcccatcagggccgggttggtaatattctacaattgggaagtaagctgattggaacaggaaaattatcagaagatgaagaaactgaagtacaagagcagatgaatctcctaaattcaagatgggaatgcctcagggtagctagcatggaaaaacaaagcaatttacatagagttttaatggatctccagaatcagaaactgaaagagttgaatgactggctaacaaaaacagaagaaagaacaaggaaaatggaggaagagcctcttggacctgatcttgaagacctaaaacgccaagtacaacaacataaggtgcttcaagaagatctagaacaagaacaagtcagggtcaattctctcactcacatggtggtggtagttgatgaatctagtggagatcacgcaactgctgctttggaagaacaacttaaggtattgggagatcgatgggcaaacatctgtagatggacagaagaccgctgggttcttttacaagacatccttctcaaatggcaacgtcttactgaagaacagtgcctttttagtgcatggctttcagaaaaagaagatgcagtgaacaagattcacacaactggctttaaagatcaaaatgaaatgttatcaagtcttcaaaaactggccgttttaaaagcggatctagaaaagaaaaagcaatccatgggcaaactgtattcactcaaacaagatcttctttcaacactgaagaataagtcagtgacccagaagacggaagcatggctggataactttgcccggtgttgggataatttagtccaaaaacttgaaaagagtacagcacagatttcacaggctgctcctggactgaccactattggagcctctcctactcagactgttactctggtgacacaacctgtggttactaaggaaactgccatctccaaactagaaatgccatcttccttgatgttggaggagctgcctcctgaggagagagcccagaatgtcactcggcttctacgaaagcaggctgaggaggtcaatactgagtgggaaaaattgaacctgcactccgctgactggcagagaaaaatagatgagacccttgaaagactccaggaacttcaagaggccacggatgagctggacctcaagctgcgccaagctgaggtgatcaagggatcctggcagcccgtgggcgatctcctcattgactctctccaagatcacctcgagaaagtcaaggcacttcgaggagaaattgcgcctctgaaagagaacgtgagccacgtcaatgaccttgctcgccagcttaccactttgggcattcagctctcaccgtataacctcagcactctggaagacctgaacaccagatggaagcttctgcaggtggccgtcgaggaccgagtcaggcagctgcatgaagcccacagggactttggtccagcatctcagcactttctttccacgtctgtccagggtccctgggagagagccatctcgccaaacaaagtgccctactatatcaaccacgagactcaaacaacttgctgggaccatcccaaaatgacagagctctaccagtctttagctgacctgaataatgtcagattctcagcttataggactgccatgaaactccgaagactgcagaaggccctttgcttggatctcttgagcctgtcagctgcatgtgatgccttggaccagcacaacctcaagcaaaatgaccagcccatggatatcctgcagattattaattgtttgaccactatttatgaccgcctggagcaagagcacaacaatttggtcaacgtccctctctgcgtggatatgtgtctgaactggctgctgaatgtttatgatacgggacgaacagggaggatccgtgtcctgtcttttaaaactggcatcatttccctgtgtaaagcacatttggaagacaagtacagataccttttcaagcaagtggcaagttcaacaggattttgtgaccagcgcaggctgggcctccttctgcatgattctatccaaattccaagacagttgggtgaagttgcatcctttgggggcagtaacattgagccaagtgtccggagctgcttccaatttgctaataataagccagagatcgaagcggccctcttcctagactggatgagactggaaccccagtccatggtgtggctgcccgtcctgcacagagtggctgctgcagaaactgccaagcatcaggccaaatgtaacatctgcaaagagtgtccaatcattggattcaggtacaggagtctaaagcactttaattatgacatctgccaaagctgctttttttctggtcgagttgcaaaaggccataaaatgcactatcccatggtggaatattgcactccgactacatcaggagaagatgttcgagactttgccaaggtactaaaaaacaaatttcgaaccaaaaggtattttgcgaagcatccccgaatgggctacctgccagtgcagactgtcttagagggggacaacatggaaactgacacaatg

SEQ ID NO: 16 - DNA, 3810 bp, Artificial Sequence
  micro-Dys5
atgctttggtgggaagaagtagaggactgttatgaaagagaagatgttcaaaagaaaacattcacaaaatgggtaaatgcacaattttctaagtttgggaagcagcatattgagaacctcttcagtgacctacaggatgggaggcgcctcctagacctcctcgaaggcctgacagggcaaaaactgccaaaagaaaaaggatccacaagagttcatgccctgaacaatgtcaacaaggcactgcgggttttgcagaacaataatgttgatttagtgaatattggaagtactgacatcgtagatggaaatcataaactgactcttggtttgatttggaatataatcctccactggcaggtcaaaaatgtaatgaaaaatatcatggctggattgcaacaaaccaacagtgaaaagattctcctgagctgggtccgacaatcaactcgtaattatccacaggttaatgtaatcaacttcaccaccagctggtctgatggcctggctttgaatgctctcatccatagtcataggccagacctatttgactggaatagtgtggtttgccagcagtcagccacacaacgactggaacatgcattcaacatcgccagatatcaattaggcatagagaaactactcgatcctgaagatgttgataccacctatccagataagaagtccatcttaatgtacatcacatcactcttccaagttttgcctcaacaagtgagcattgaagccatccaggaagtggaaatgttgccaaggccacctaaagtgactaaagaagaacattttcagttacatcatcaaatgcactattctcaacagatcacggtcagtctagcacagggatatgagagaacttcttcccctaagcctcgattcaagagctatgcctacacacaggctgcttatgtcaccacctctgaccctacacggagcccatttccttcacagcatttggaagctcctgaagacaagtcatttggcagttcattgatggagagtgaagtaaacctggaccgttatcaaacagctttagaagaagtattatcgtggcttctttctgctgaggacacattgcaagcacaaggagagatttctaatgatgtggaagtggtgaaagaccagtttcatactcatgaggggtacatgatggatttgacagcccatcagggccgggttggtaatattctacaattgggaagtaagctgattggaacaggaaaattatcagaagatgaagaaactgaagtacaagagcagatgaatctcctaaattcaagatgggaatgcctcagggtagctagcatggaaaaacaaagcaatttacattcttatgtgccttctacttatttgactgaaatcactcatgtctcacaagccctattagaagtggaacaacttctcaatgctcctgacctctgtgctaaggactttgaagatctctttaagcaagaggagtctctgaagaatataaaagatagtctacaacaaagctcaggtcggattgacattattcatagcaagaagacagcagcattgcaaagtgcaacgcctgtggaaagggtgaagctacaggaagctctctcccagcttgatttccaatgggaaaaagttaacaaaatgtacaaggaccgacaagggcgatttgacagatctgttgagaaatggcggcgttttcattatgatataaagatatttaatcagtggctaacagaagctgaacagtttctcagaaagacacaaattcctgagaattgggaacatgctaaatacaaatggtatcttaaggaactccaggatggcattgggcagcggcaaactgttgtcagaacattgaatgcaactggggaagaaataattcagcaatcctcaaaaacagatgccagtattctacaggaaaaattgggaagcctgaatctgcggtggcaggaggtctgcaaacagctgtcagacagaaaaaagaggctagaagaacaatctgaccagtggaagcgtctgcacctttctctgcaggaacttctggtgtggctacagctgaaagatgatgaattaagccggcaggcacctattggaggcgactttccagcagttcagaagcagaacgatgtacatagggccttcaagagggaattgaaaactaaagaacctgtaatcatgagtactcttgagactgtacgaatatttctgacagagcagcctttggaaggactagagaaactctaccaggagcccagagagctgcctcctgaggagagagcccagaatgtcactcggcttctacgaaagcaggctgaggaggtcaatactgagtgggaaaaattgaacctgcactccgctgactggcagagaaaaatagatgagacccttgaaagactccaggaacttcaagaggccacggatgagctggacctcaagctgcgccaagctgaggtgatcaagggatcctggcagcccgtgggcgatctcctcattgactctctccaagatcacctcgagaaagtcaaggcacttcgaggagaaattgcgcctctgaaagagaacgtgagccacgtcaatgaccttgctcgccagcttaccactttgggcattcagctctcaccgtataacctcagcactctggaagacctgaacaccagatggaagcttctgcaggtggccgtcgaggaccgagtcaggcagctgcatgaagcccacagggactttggtccagcatctcagcactttctttccacgtctgtccagggtccctgggagagagccatctcgccaaacaaagtgccctactatatcaaccacgagactcaaacaacttgctgggaccatcccaaaatgacagagctctaccagtctttagctgacctgaataatgtcagattctcagcttataggactgccatgaaactccgaagactgcagaaggccctttgcttggatctcttgagcctgtcagctgcatgtgatgccttggaccagcacaacctcaagcaaaatgaccagcccatggatatcctgcagattattaattgtttgaccactatttatgaccgcctggagcaagagcacaacaatttggtcaacgtccctctctgcgtggatatgtgtctgaactggctgctgaatgtttatgatacgggacgaacagggaggatccgtgtcctgtcttttaaaactggcatcatttccctgtgtaaagcacatttggaagacaagtacagataccttttcaagcaagtggcaagttcaacaggattttgtgaccagcgcaggctgggcctccttctgcatgattctatccaaattccaagacagttgggtgaagttgcatcctttgggggcagtaacattgagccaagtgtccggagctgcttccaatttgctaataataagccagagatcgaagcggccctcttcctagactggatgagactggaaccccagtccatggtgtggctgcccgtcctgcacagagtggctgctgcagaaactgccaagcatcaggccaaatgtaacatctgcaaagagtgtccaatcattggattcaggtacaggagtctaaagcactttaattatgacatctgccaaagctgctttttttctggtcgagttgcaaaaggccataaaatgcactatcccatggtggaatattgcactccgactacatcaggagaagatgttcgagactttgccaaggtactaaaaaacaaatttcgaaccaaaaggtattttgcgaagcatccccgaatgggctacctgccagtgcagactgtcttagagggggacaacatggaaactgacacaatg

SEQ ID NO: 17 - DNA, 4149 bp, Artificial Sequence
  micro-Dys6
atgctttggtgggaagaagtagaggactgttatgaaagagaagatgttcaaaagaaaacattcacaaaatgggtaaatgcacaattttctaagtttgggaagcagcatattgagaacctcttcagtgacctacaggatgggaggcgcctcctagacctcctcgaaggcctgacagggcaaaaactgccaaaagaaaaaggatccacaagagttcatgccctgaacaatgtcaacaaggcactgcgggttttgcagaacaataatgttgatttagtgaatattggaagtactgacatcgtagatggaaatcataaactgactcttggtttgatttggaatataatcctccactggcaggtcaaaaatgtaatgaaaaatatcatggctggattgcaacaaaccaacagtgaaaagattctcctgagctgggtccgacaatcaactcgtaattatccacaggttaatgtaatcaacttcaccaccagctggtctgatggcctggctttgaatgctctcatccatagtcataggccagacctatttgactggaatagtgtggtttgccagcagtcagccacacaacgactggaacatgcattcaacatcgccagatatcaattaggcatagagaaactactcgatcctgaagatgttgataccacctatccagataagaagtccatcttaatgtacatcacatcactcttccaagttttgcctcaacaagtgagcattgaagccatccaggaagtggaaatgttgccaaggccacctaaagtgactaaagaagaacattttcagttacatcatcaaatgcactattctcaacagatcacggtcagtctagcacagggatatgagagaacttcttcccctaagcctcgattcaagagctatgcctacacacaggctgcttatgtcaccacctctgaccctacacggagcccatttccttcacagcatttggaagctcctgaagacaagtcatttggcagttcattgatggagagtgaagtaaacctggaccgttatcaaacagctttagaagaagtattatcgtggcttctttctgctgaggacacattgcaagcacaaggagagatttctaatgatgtggaagtggtgaaagaccagtttcatactcatgaggggtacatgatggatttgacagcccatcagggccgggttggtaatattctacaattgggaagtaagctgattggaacaggaaaattatcagaagatgaagaaactgaagtacaagagcagatgaatctcctaaattcaagatgggaatgcctcagggtagctagcatggaaaaacaaagcaatttacatagagttttaatggatctccagaatcagaaactgaaagagttgaatgactggctaacaaaaacagaagaaagaacaaggaaaatggaggaagagcctcttggacctgatcttgaagacctaaaacgccaagtacaacaacataaggtgcttcaagaagatctagaacaagaacaagtcagggtcaattctctcactcacatggtggtggtagttgatgaatctagtggagatcacgcaactgctgctttggaagaacaacttaaggtattgggagatcgatgggcaaacatctgtagatggacagaagaccgctgggttcttttacaagacatccttctcaaatggcaacgtcttactgaagaacagtgcctttttagtgcatggctttcagaaaaagaagatgcagtgaacaagattcacacaactggctttaaagatcaaaatgaaatgttatcaagtcttcaaaaactggccgttttaaaagcggatctagaaaagaaaaagcaatccatgggcaaactgtattcactcaaacaagatcttctttcaacactgaagaataagtcagtgacccagaagacggaagcatggctggataactttgcccggtgttgggataatttagtccaaaaacttgaaaagagtacagcacagatttcacaggctattcacactgtccgtgaagaaacgatgatggtgatgactgaagacatgcctttggaaatttcttatgtgccttctacttatttgactgaaatcactcatgtctcacaagccctattagaagtggaacaacttctcaatgctcctgacctctgtgctaaggactttgaagatctctttaagcaagaggagtctctgaagaatataaaagatagtctacaacaaagctcaggtcggattgacattattcatagcaagaagacagcagcattgcaaagtgcaacgcctgtggaaagggtgaagctacaggaagctctctcccagcttgatttccaatgggaaaaagttaacaaaatgtacaaggaccgacaagggcgatttgacagatctgttgagaaatggcggcgttttcattatgatataaagatatttaatcagtggctaacagaagctgaacagtttctcagaaagacacaaattcctgagaattgggaacatgctaaatacaaatggtatcttaaggaactccaggatggcattgggcagcggcaaactgttgtcagaacattgaatgcaactggggaagaaataattcagcaatcctcaaaaacagatgccagtattctacaggaaaaattgggaagcctgaatctgcggtggcaggaggtctgcaaacagctgtcagacagaaaaaagaggctagaagaacaacttgaaagactccaggaacttcaagaggccacggatgagctggacctcaagctgcgccaagctgaggtgatcaagggatcctggcagcccgtgggcgatctcctcattgactctctccaagatcacctcgagaaagtcaaggcacttcgaggagaaattgcgcctctgaaagagaacgtgagccacgtcaatgaccttgctcgccagcttaccactttgggcattcagctctcaccgtataacctcagcactctggaagacctgaacaccagatggaagcttctgcaggtggccgtcgaggaccgagtcaggcagctgcatgaagcccacagggactttggtccagcatctcagcactttctttccacgtctgtccagggtccctgggagagagccatctcgccaaacaaagtgccctactatatcaaccacgagactcaaacaacttgctgggaccatcccaaaatgacagagctctaccagtctttagctgacctgaataatgtcagattctcagcttataggactgccatgaaactccgaagactgcagaaggccctttgcttggatctcttgagcctgtcagctgcatgtgatgccttggaccagcacaacctcaagcaaaatgaccagcccatggatatcctgcagattattaattgtttgaccactatttatgaccgcctggagcaagagcacaacaatttggtcaacgtccctctctgcgtggatatgtgtctgaactggctgctgaatgtttatgatacgggacgaacagggaggatccgtgtcctgtcttttaaaactggcatcatttccctgtgtaaagcacatttggaagacaagtacagataccttttcaagcaagtggcaagttcaacaggattttgtgaccagcgcaggctgggcctccttctgcatgattctatccaaattccaagacagttgggtgaagttgcatcctttgggggcagtaacattgagccaagtgtccggagctgcttccaatttgctaataataagccagagatcgaagcggccctcttcctagactggatgagactggaaccccagtccatggtgtggctgcccgtcctgcacagagtggctgctgcagaaactgccaagcatcaggccaaatgtaacatctgcaaagagtgtccaatcattggattcaggtacaggagtctaaagcactttaattatgacatctgccaaagctgctttttttctggtcgagttgcaaaaggccataaaatgcactatcccatggtggaatattgcactccgactacatcaggagaagatgttcgagactttgccaaggtactaaaaaacaaatttcgaaccaaaaggtattttgcgaagcatccccgaatgggctacctgccagtgcagactgtcttagagggggacaacatggaaactgacacaatg

SEQ ID NO: 18 - DNA, 4212 bp, Artificial Sequence
  micro-Dys7
atgctttggtgggaagaagtagaggactgttatgaaagagaagatgttcaaaagaaaacattcacaaaatgggtaaatgcacaattttctaagtttgggaagcagcatattgagaacctcttcagtgacctacaggatgggaggcgcctcctagacctcctcgaaggcctgacagggcaaaaactgccaaaagaaaaaggatccacaagagttcatgccctgaacaatgtcaacaaggcactgcgggttttgcagaacaataatgttgatttagtgaatattggaagtactgacatcgtagatggaaatcataaactgactcttggtttgatttggaatataatcctccactggcaggtcaaaaatgtaatgaaaaatatcatggctggattgcaacaaaccaacagtgaaaagattctcctgagctgggtccgacaatcaactcgtaattatccacaggttaatgtaatcaacttcaccaccagctggtctgatggcctggctttgaatgctctcatccatagtcataggccagacctatttgactggaatagtgtggtttgccagcagtcagccacacaacgactggaacatgcattcaacatcgccagatatcaattaggcatagagaaactactcgatcctgaagatgttgataccacctatccagataagaagtccatcttaatgtacatcacatcactcttccaagttttgcctcaacaagtgagcattgaagccatccaggaagtggaaatgttgccaaggccacctaaagtgactaaagaagaacattttcagttacatcatcaaatgcactattctcaacagatcacggtcagtctagcacagggatatgagagaacttcttcccctaagcctcgattcaagagctatgcctacacacaggctgcttatgtcaccacctctgaccctacacggagcccatttccttcacagcatttggaagctcctgaagacaagtcatttggcagttcattgatggagagtgaagtaaacctggaccgttatcaaacagctttagaagaagtattatcgtggcttctttctgctgaggacacattgcaagcacaaggagagatttctaatgatgtggaagtggtgaaagaccagtttcatactcatgaggggtacatgatggatttgacagcccatcagggccgggttggtaatattctacaattgggaagtaagctgattggaacaggaaaattatcagaagatgaagaaactgaagtacaagagcagatgaatctcctaaattcaagatgggaatgcctcagggtagctagcatggaaaaacaaagcaatttacatagagttttaatggatctccagaatcagaaactgaaagagttgaatgactggctaacaaaaacagaagaaagaacaaggaaaatggaggaagagcctcttggacctgatcttgaagacctaaaacgccaagtacaacaacataaggtgcttcaagaagatctagaacaagaacaagtcagggtcaattctctcactcacatggtggtggtagttgatgaatctagtggagatcacgcaactgctgctttggaagaacaacttaaggtattgggagatcgatgggcaaacatctgtagatggacagaagaccgctgggttcttttacaagacatccttctcaaatggcaacgtcttactgaagaacagtgcctttttagtgcatggctttcagaaaaagaagatgcagtgaacaagattcacacaactggctttaaagatcaaaatgaaatgttatcaagtcttcaaaaactggccgttttaaaagcggatctagaaaagaaaaagcaatccatgggcaaactgtattcactcaaacaagatcttctttcaacactgaagaataagtcagtgacccagaagacggaagcatggctggataactttgcccggtgttgggataatttagtccaaaaacttgaaaagagtacagcacagatttcacaggctgctcctggactgaccactattggagcctctcctactcagactgttactctggtgacacaacctgtggttactaaggaaactgccatctccaaactagaaatgccatcttccttgatgttggagtcttatgtgccttctacttatttgactgaaatcactcatgtctcacaagccctattagaagtggaacaacttctcaatgctcctgacctctgtgctaaggactttgaagatctctttaagcaagaggagtctctgaagaatataaaagatagtctacaacaaagctcaggtcggattgacattattcatagcaagaagacagcagcattgcaaagtgcaacgcctgtggaaagggtgaagctacaggaagctctctcccagcttgatttccaatgggaaaaagttaacaaaatgtacaaggaccgacaagggcgatttgacagatctgttgagaaatggcggcgttttcattatgatataaagatatttaatcagtggctaacagaagctgaacagtttctcagaaagacacaaattcctgagaattgggaacatgctaaatacaaatggtatcttaaggaactccaggatggcattgggcagcggcaaactgttgtcagaacattgaatgcaactggggaagaaataattcagcaatcctcaaaaacagatgccagtattctacaggaaaaattgggaagcctgaatctgcggtggcaggaggtctgcaaacagctgtcagacagaaaaaagaggctagaagaacaacttgaaagactccaggaacttcaagaggccacggatgagctggacctcaagctgcgccaagctgaggtgatcaagggatcctggcagcccgtgggcgatctcctcattgactctctccaagatcacctcgagaaagtcaaggcacttcgaggagaaattgcgcctctgaaagagaacgtgagccacgtcaatgaccttgctcgccagcttaccactttgggcattcagctctcaccgtataacctcagcactctggaagacctgaacaccagatggaagcttctgcaggtggccgtcgaggaccgagtcaggcagctgcatgaagcccacagggactttggtccagcatctcagcactttctttccacgtctgtccagggtccctgggagagagccatctcgccaaacaaagtgccctactatatcaaccacgagactcaaacaacttgctgggaccatcccaaaatgacagagctctaccagtctttagctgacctgaataatgtcagattctcagcttataggactgccatgaaactccgaagactgcagaaggccctttgcttggatctcttgagcctgtcagctgcatgtgatgccttggaccagcacaacctcaagcaaaatgaccagcccatggatatcctgcagattattaattgtttgaccactatttatgaccgcctggagcaagagcacaacaatttggtcaacgtccctctctgcgtggatatgtgtctgaactggctgctgaatgtttatgatacgggacgaacagggaggatccgtgtcctgtcttttaaaactggcatcatttccctgtgtaaagcacatttggaagacaagtacagataccttttcaagcaagtggcaagttcaacaggattttgtgaccagcgcaggctgggcctccttctgcatgattctatccaaattccaagacagttgggtgaagttgcatcctttgggggcagtaacattgagccaagtgtccggagctgcttccaatttgctaataataagccagagatcgaagcggccctcttcctagactggatgagactggaaccccagtccatggtgtggctgcccgtcctgcacagagtggctgctgcagaaactgccaagcatcaggccaaatgtaacatctgcaaagagtgtccaatcattggattcaggtacaggagtctaaagcactttaattatgacatctgccaaagctgctttttttctggtcgagttgcaaaaggccataaaatgcactatcccatggtggaatattgcactccgactacatcaggagaagatgttcgagactttgccaaggtactaaaaaacaaatttcgaaccaaaaggtattttgcgaagcatccccgaatgggctacctgccagtgcagactgtcttagagggggacaacatggaaactgacacaatg

SEQ ID NO: 19 - DNA, 450 bp, Artificial Sequence
  CK8 promoter
ctagactagcatgctgcccatgtaaggaggcaaggcctggggacacccgagatgcctggttataattaacccagacatgtggctgcccccccccccccaacacctgctgcctctaaaaataaccctgcatgccatgttcccggcgaagggccagctgtcccccgccagctagactcagcacttagtttaggaaccagtgagcaagtcagcccttggggcagcccatacaaggccatggggctgggcaagctgcacgcctgggtccggggtgggcacggtgcccgggcaacgagctgaaagctcatctgctctcaggggcccctccctggggacagcccctcctggctagtcacaccctgtaggctcctctatataacccaggggcacaggggctgccctcattctaccaccacctccacagcacagacagacactcaggagccagccagc

SEQ ID NO: 20 - protein, 20 aa, Artificial Sequence
  Hinge-like region between SR15 and SR16
IHTVREETMMVMTEDMPLEI

SEQ ID NO: 21 - protein, 20 aa, Artificial Sequence
  Hinge-like region within SR23
LEGLEKLYQEPRELPPEERA

SEQ ID NO: 22 - DNA, 8391 bp, Artificial Sequence
  CK8-micro-Dys5 cassette
cagcagctgcgcgctcgctcgctcactgaggccgcccgggcaaagcccgggcgtcgggcgacctttggtcgcccggcctcagtgagcgagcgagcgcgcagagagggagtggccaactccatcactaggggttccttgtagttaatgattaacccgccatgctacttatctacaaacgctagcatgctgcccatgtaaggaggcaaggcctggggacacccgagatgcctggttataattaacccagacatgtggctgcccccccccccccaacacctgctgcctctaaaaataaccctgcatgccatgttcccggcgaagggccagctgtcccccgccagctagactcagcacttagtttaggaaccagtgagcaagtcagcccttggggcagcccatacaaggccatggggctgggcaagctgcacgcctgggtccggggtgggcacggtgcccgggcaacgagctgaaagctcatctgctctcaggggcccctccctggggacagcccctcctggctagtcacaccctgtaggctcctctatataacccaggggcacaggggctgccctcattctaccaccacctccacagcacagacagacactcaggagccagccagcgtcgaggttaacccgcggccgttttttttatcgctgccttgatatacactttccaccatgctttggtgggaagaagtagaggactgttatgaaagagaagatgttcaaaagaaaacattcacaaaatgggtaaatgcacaattttctaagtttgggaagcagcatattgagaacctcttcagtgacctacaggatgggaggcgcctcctagacctcctcgaaggcctgacagggcaaaaactgccaaaagaaaaaggatccacaagagttcatgccctgaacaatgtcaacaaggcactgcgggttttgcagaacaataatgttgatttagtgaatattggaagtactgacatcgtagatggaaatcataaactgactcttggtttgatttggaatataatcctccactggcaggtcaaaaatgtaatgaaaaatatcatggctggattgcaacaaaccaacagtgaaaagattctcctgagctgggtccgacaatcaactcgtaattatccacaggttaatgtaatcaacttcaccaccagctggtctgatggcctggctttgaatgctctcatccatagtcataggccagacctatttgactggaatagtgtggtttgccagcagtcagccacacaacgactggaacatgcattcaacatcgccagatatcaattaggcatagagaaactactcgatcctgaagatgttgataccacctatccagataagaagtccatcttaatgtacatcacatcactcttccaagttttgcctcaacaagtgagcattgaagccatccaggaagtggaaatgttgccaaggccacctaaagtgactaaagaagaacattttcagttacatcatcaaatgcactattctcaacagatcacggtcagtctagcacagggatatgagagaacttcttcccctaagcctcgattcaagagctatgcctacacacaggctgcttatgtcaccacctctgaccctacacggagcccatttccttcacagcatttggaagctcctgaagacaagtcatttggcagttcattgatggagagtgaagtaaacctggaccgttatcaaacagctttagaagaagtattatcgtggcttctttctgctgaggacacattgcaagcacaaggagagatttctaatgatgtggaagtggtgaaagaccagtttcatactcatgaggggtacatgatggatttgacagcccatcagggccgggttggtaatattctacaattgggaagtaagctgattggaacaggaaaattatcagaagatgaagaaactgaagtacaagagcagatgaatctcctaaattcaagatgggaatgcctcagggtagctagcatggaaaaacaaagcaatttacattcttatgtgccttctacttatttgactgaaatcactcatgtctcacaagccctattagaagtggaacaacttctcaatgctcctgacctctgtgctaaggactttgaagatctctttaagcaagaggagtctctgaagaatataaaagatagtctacaacaaagctcaggtcggattgacattattcatagcaagaagacagcagcattgcaaagtgcaacgcctgtggaaagggtgaagctacaggaagctctctcccagcttgatttccaatgggaaaaagttaacaaaatgtacaaggaccgacaagggcgatttgacagatctgttgagaaatggcggcgttttcattatgatataaagatatttaatcagtggctaacagaagctgaacagtttctcagaaagacacaaattcctgagaattgggaacatgctaaatacaaatggtatcttaaggaactccaggatggcattgggcagcggcaaactgttgtcagaacattgaatgcaactggggaagaaataattcagcaatcctcaaaaacagatgccagtattctacaggaaaaattgggaagcctgaatctgcggtggcaggaggtctgcaaacagctgtcagacagaaaaaagaggctagaagaacaatctgaccagtggaagcgtctgcacctttctctgcaggaacttctggtgtggctacagctgaaagatgatgaattaagccggcaggcacctattggaggcgactttccagcagttcagaagcagaacgatgtacatagggccttcaagagggaattgaaaactaaagaacctgtaatcatgagtactcttgagactgtacgaatatttctgacagagcagcctttggaaggactagagaaactctaccaggagcccagagagctgcctcctgaggagagagcccagaatgtcactcggcttctacgaaagcaggctgaggaggtcaatactgagtgggaaaaattgaacctgcactccgctgactggcagagaaaaatagatgagacccttgaaagactccaggaacttcaagaggccacggatgagctggacctcaagctgcgccaagctgaggtgatcaagggatcctggcagcccgtgggcgatctcctcattgactctctccaagatcacctcgagaaagtcaaggcacttcgaggagaaattgcgcctctgaaagagaacgtgagccacgtcaatgaccttgctcgccagcttaccactttgggcattcagctctcaccgtataacctcagcactctggaagacctgaacaccagatggaagcttctgcaggtggccgtcgaggaccgagtcaggcagctgcatgaagcccacagggactttggtccagcatctcagcactttctttccacgtctgtccagggtccctgggagagagccatctcgccaaacaaagtgccctactatatcaaccacgagactcaaacaacttgctgggaccatcccaaaatgacagagctctaccagtctttagctgacctgaataatgtcagattctcagcttataggactgccatgaaactccgaagactgcagaaggccctttgcttggatctcttgagcctgtcagctgcatgtgatgccttggaccagcacaacctcaagcaaaatgaccagcccatggatatcctgcagattattaattgtttgaccactatttatgaccgcctggagcaagagcacaacaatttggtcaacgtccctctctgcgtggatatgtgtctgaactggctgctgaatgtttatgatacgggacgaacagggaggatccgtgtcctgtcttttaaaactggcatcatttccctgtgtaaagcacatttggaagacaagtacagataccttttcaagcaagtggcaagttcaacaggattttgtgaccagcgcaggctgggcctccttctgcatgattctatccaaattccaagacagttgggtgaagttgcatcctttgggggcagtaacattgagccaagtgtccggagctgcttccaatttgctaataataagccagagatcgaagcggccctcttcctagactggatgagactggaaccccagtccatggtgtggctgcccgtcctgcacagagtggctgctgcagaaactgccaagcatcaggccaaatgtaacatctgcaaagagtgtccaatcattggattcaggtacaggagtctaaagcactttaattatgacatctgccaaagctgctttttttctggtcgagttgcaaaaggccataaaatgcactatcccatggtggaatattgcactccgactacatcaggagaagatgttcgagactttgccaaggtactaaaaaacaaatttcgaaccaaaaggtattttgcgaagcatccccgaatgggctacctgccagtgcagactgtcttagagggggacaacatggaaactgacacaatgtaggaagtcttttccacatggcagatgaaccggtggctagtaataaaagatccttattttcattggatctgtgtgttggttttttgtgtgggtaccgtttgtagataagtagcatggcgggttaatcattaactacaaggaacccctagtgatggagttggccactccctctctgcgcgctcgctcgctcactgaggccgggcgaccaaaggtcgcccgacgcccgggctttgcccgggcggcctcagtgagcgagcgagcgcgccagctggcgtaatagcgaagaggcccgcaccgatcgcccttcccaacagttgcgcagcctgaatggcgaatggaattccagacgattgagcgtcaaaatgtaggtatttccatgagcgtttttcctgttgcaatggctggcggtaatattgttctggatattaccagcaaggccgatagtttgagttcttctactcaggcaagtgatgttattactaatcaaagaagtattgcgacaacggttaatttgcgtgatggacagactcttttactcggtggcctcactgattataaaaacacttctcaggattctggcgtaccgttcctgtctaaaatccctttaatcggcctcctgtttagctcccgctctgattctaacgaggaaagcacgttatacgtgctcgtcaaagcaaccatagtacgcgccctgtagcggcgcattaagcgcggcgggtgtggtggttacgcgcagcgtgaccgctacacttgccagcgccctagcgcccgctcctttcgctttcttcccttcctttctcgccacgttcgccggctttccccgtcaagctctaaatcgggggctccctttagggttccgatttagtgctttacggcacctcgaccccaaaaaacttgattagggtgatggttcacgtagtgggccatcgccctgatagacggtttttcgccctttgacgttggagtccacgttctttaatagtggactcttgttccaaactggaacaacactcaaccctatctcggtctattcttttgatttataagggattttgccgatttcggcctattggttaaaaaatgagctgatttaacaaaaatttaacgcgaattttaacaaaatattaacgtttacaatttaaatatttgcttatacaatcttcctgtttttggggcttttctgattatcaaccggggtacatatgattgacatgctagttttacgattaccgttcatcgattctcttgtttgctccagactctcaggcaatgacctgatagcctttgtagagacctctcaaaaatagctaccctctccggcatgaatttatcagctagaacggttgaatatcatattgatggtgatttgactgtctccggcctttctcacccgtttgaatctttacctacacattactcaggcattgcatttaaaatatatgagggttctaaaaatttttatccttgcgttgaaataaaggcttctcccgcaaaagtattacagggtcataatgtttttggtacaaccgatttagctttatgctctgaggctttattgcttaattttgctaattctttgccttgcctgtatgatttattggatgttggaattcctgatgcggtattttctccttacgcatctgtgcggtatttcacaccgcatatggtgcactctcagtacaatctgctctgatgccgcatagttaagccagccccgacacccgccaacacccgctgacgcgccctgacgggcttgtctgctcccggcatccgcttacagacaagctgtgaccgtctccgggagctgcatgtgtcagaggttttcaccgtcatcaccgaaacgcgcgagacgaaagggcctcgtgatacgcctatttttataggttaatgtcatgataataatggtttcttagacgtcaggtggcacttttcggggaaatgtgcgcggaacccctatttgtttatttttctaaatacattcaaatatgtatccgctcatgagacaataaccctgataaatgcttcaataatattgaaaaaggaagagtatgagtattcaacatttccgtgtcgcccttattcccttttttgcggcattttgccttcctgtttttgctcacccagaaacgctggtgaaagtaaaagatgctgaagatcagttgggtgcacgagtgggttacatcgaactggatctcaacagcggtaagatccttgagagttttcgccccgaagaacgttttccaatgatgagcacttttaaagttctgctatgtggcgcggtattatcccgtattgacgccgggcaagagcaactcggtcgccgcatacactattctcagaatgacttggttgagtactcaccagtcacagaaaagcatcttacggatggcatgacagtaagagaattatgcagtgctgccataaccatgagtgataacactgcggccaacttacttctgacaacgatcggaggaccgaaggagctaaccgcttttttgcacaacatgggggatcatgtaactcgccttgatcgttgggaaccggagctgaatgaagccataccaaacgacgagcgtgacaccacgatgcctgtagcaatggcaacaacgttgcgcaaactattaactggcgaactacttactctagcttcccggcaacaattaatagactggatggaggcggataaagttgcaggaccacttctgcgctcggcccttccggctggctggtttattgctgataaatctggagccggtgagcgtgggtctcgcggtatcattgcagcactggggccagatggtaagccctcccgtatcgtagttatctacacgacggggagtcaggcaactatggatgaacgaaatagacagatcgctgagataggtgcctcactgattaagcattggtaactgtcagaccaagtttactcatatatactttagattgatttaaaacttcatttttaatttaaaaggatctaggtgaagatcctttttgataatctcatgaccaaaatcccttaacgtgagttttcgttccactgagcgtcagaccccgtagaaaagatcaaaggatcttcttgagatcctttttttctgcgcgtaatctgctgcttgcaaacaaaaaaaccaccgctaccagcggtggtttgtttgccggatcaagagctaccaactctttttccgaaggtaactggcttcagcagagcgcagataccaaatactgtccttctagtgtagccgtagttaggccaccacttcaagaactctgtagcaccgcctacatacctcgctctgctaatcctgttaccagtggctgctgccagtggcgataagtcgtgtcttaccgggttggactcaagacgatagttaccggataaggcgcagcggtcgggctgaacggggggttcgtgcacacagcccagcttggagcgaacgacctacaccgaactgagatacctacagcgtgagctatgagaaagcgccacgcttcccgaagggagaaaggcggacaggtatccggtaagcggcagggtcggaacaggagagcgcacgagggagcttccagggggaaacgcctggtatctttatagtcctgtcgggtttcgccacctctgacttgagcgtcgatttttgtgatgctcgtcaggggggcggagcctatggaaaaacgccagcaacgcggcctttttacggttcctggccttttgctggccttttgctcacatgttctttcctgcgttatcccctgattctgtggataaccgtattaccgcctttgagtgagctgataccgctcgccgcagccgaacgaccgagcgcagcgagtcagtgagcgaggaagcggaagagcgcccaatacgcaaaccgcctctccccgcgcgttggccgattcattaatg